European Patent Application EP 4 202 035 A1, published June 28, 2023. Title: Verbesserter CP45 Produktionsstamm. Applicant: Gelita AG. The sequence listing filed with the application follows.

SEQUENCE LISTING (26 sequences)

SEQ ID NO: 1 - DNA, 1551 bp, Artificial Sequence
  codon optimized 45 kDa Col1A1
gagcgtggatttccaggcgaaaggggtgttcaaggcccacctggtcctgctggcccaagaggtgctaatggtgctcctggtaatgatggcgctaaaggtgacgccggtgctcccggtgcacccggttctcaaggtgcccctggcttgcaaggtatgccaggcgagcgtggtgctgctggattgcctggaccaaagggcgatagaggtgatgccggtccaaagggtgctgacggtgcaccaggtaaggacggtgtaagaggtttgactggacctattggccctccaggtccagccggtgcaccaggcgataagggtgaagctggaccttccggtccagctggccctactggtgctagaggtgccccaggtgatagaggcgagcctggtcctcctggacctgcaggctttgctggtcctcctggtgctgatggtcaacctggtgccaagggtgagccaggtgatgctggcgccaaaggtgatgcaggcccacctggacctgccggtcctgccggacctccaggtcctattggtaatgttggtgctcccggacctaaaggcgctagaggttcagccggtcctccaggcgctactggtttccctggtgctgcaggtagagttggtccaccaggtccatctggtaatgcaggaccaccaggtcctccaggtccagccggtaaagaaggttctaaaggtcctaggggtgaaactggtcccgcaggtaggcccggtgaagtaggccctccaggtcctcctggaccagctggcgaaaaaggtgctcctggcgcagatggtcctgccggcgctcctggaactccaggacctcagggtattgctggacaaagaggtgttgttggtctgccaggtcaacgtggtgaaagaggctttccaggactgcctggtccatcaggcgagccaggtaagcaaggaccatccggtgcttcaggcgaaagaggcccaccaggaccaatgggtccacctggtttagcaggacctccaggcgaatctggtagagaaggcgcaccaggcgctgaaggttctccaggtagagatggaagtcctggcgctaagggcgatcgtggcgaaactggccccgctggacctccaggcgctccaggtgctcccggcgctccaggaccagtcggtccagccggcaaatctggtgatagaggtgaaacaggcccagctggcccagccggaccaatcggtcctgttggtgctaggggtcccgctggtcctcaaggaccaaggggtgacaagggtgaaaccggtgaacagggtgatcgtggtattaagggacaccgtggattttccggattgcaaggacctcctggtcctccaggatctcccggtgaacaaggaccttctggtgcatctggacccgcaggacccaggggtccaccaggatctgctggaagtccaggtaaggatggtttgaacggtttgccaggaccaatcggccctcctggaccaagaggtagaactggtgatgccggaccagccggtccaccaggaccacctggacctccaggacctcctggtcctccttcttaa

SEQ ID NO: 2 - protein, 516 aa, Artificial Sequence
  45 kDa Col1A1 fragment
ERGFPGERGVQGPPGPAGPRGANGAPGNDGAKGDAGAPGAPGSQGAPGLQGMPGERGAAGLPGPKGDRGDAGPKGADGAPGKDGVRGLTGPIGPPGPAGAPGDKGEAGPSGPAGPTGARGAPGDRGEPGPPGPAGFAGPPGADGQPGAKGEPGDAGAKGDAGPPGPAGPAGPPGPIGNVGAPGPKGARGSAGPPGATGFPGAAGRVGPPGPSGNAGPPGPPGPAGKEGSKGPRGETGPAGRPGEVGPPGPPGPAGEKGAPGADGPAGAPGTPGPQGIAGQRGVVGLPGQRGERGFPGLPGPSGEPGKQGPSGASGERGPPGPMGPPGLAGPPGESGREGAPGAEGSPGRDGSPGAKGDRGETGPAGPPGAPGAPGAPGPVGPAGKSGDRGETGPAGPAGPIGPVGARGPAGPQGPRGDKGETGEQGDRGIKGHRGFSGLQGPPGPPGSPGEQGPSGASGPAGPRGPPGSAGSPGKDGLNGLPGPIGPPGPRGRTGDAGPAGPPGPPGPPGPPGPPS

SEQ ID NO: 3 - DNA, 47 bp, Artificial Sequence
  forward Primer GE34
tcgagaagagagaggccgaagctgagcgtggatttccaggcgaaagg

SEQ ID NO: 4 - DNA, 47 bp, Artificial Sequence
  reverse Primer GE35
ttctgacatcctcttgattaagaaggaggaccaggaggtcctggagg

SEQ ID NO: 5 - DNA, 21 bp, Artificial Sequence
  forward Primer GE36
atgagattcccatctattttc

SEQ ID NO: 6 - DNA, 18 bp, Artificial Sequence
  reverse Primer GE37
acatgtgagcaaaaggcc

SEQ ID NO: 7 - DNA, 38 bp, Artificial Sequence
  forward Primer GE40
ctggccttttgctcacatgttaatcgaactccgaatgc

SEQ ID NO: 8 - DNA, 47 bp, Artificial Sequence
  reverse Primer GE41
gtgaaaatagatgggaatctcattttaattgtaagtcttgactagag

SEQ ID NO: 9 - DNA, 4035 bp, Artificial Sequence
  pBSYGAPsec_blunt1
  misc_feature (1)..(8): linearization site
  promoter (9)..(494): PGAP
  sig_peptide (495)..(761): MatAlpha
  misc_feature (762)..(1588): Stuffer MlyI Cloning
  terminator (1592)..(1851): AOX1TT
  source (1857)..(1858)
  promoter (1859)..(2416): PILV5
  promoter (2417)..(2480): PEM72
  misc_feature (2482)..(2856): ZeoR
  terminator (2858)..(3333): AODTT
  rep_origin (3360)..(4030): pUC ORI
atttaaattttttgtagaaatgtcttggtgtcctcgtccaatcaggtagccatctctgaaatatctggctccgttgcaactccgaacgacctgctggcaacgtaaaattctccggggtaaaacttaaatgtggagtaatggaaccagaaacgtctcttcccttctctctccttccaccgcccgttaccgtccctaggaaattttactctgctggagagcttcttctacggcccccttgcagcaatgctcttcccagcattacgttgcgggtaaaacggaggtcgtgtacccgacctagcagcccagggatggaaaagtcccggccgtcgctggcaataatagcgggcggacgcatgtcatgagattattggaaaccaccagaatcgaatataaaaggcgaacacctttcccaattttggtttctcctgacccaaagactttaaatttaatttatttgtccctatttcaatcaattgaacaactatcaaaacacaatgagattcccatctattttcaccgctgtcttgttcgctgcctcctctgcattggctgcccctgttaacactaccactgaagacgagactgctcaaattccagctgaagcagttatcggttactctgaccttgagggtgatttcgacgtcgctgttttgcctttctctaactccactaacaacggtttgttgttcattaacaccactatcgcttccattgctgctaaggaagagggtgtctctctcgagaagagagaggccgaagctctgaggactcgaattcgacctctgttgcctctttgttggacgaaccattcaccggtgtcttgtacttaaagggcagtggtatcactgaagacttccagtccctaaagggtaagaagatcggttacgttggtgacttcggtaagatccaaatcgatgaattgaccaagcactacggtatgaagccagaagactacaccgccgtcagatgtggtatgaatgtcgccaagtacatcatcgaaggtaagattgatgccggtattggtatcgaatgtatgcaacaagtcgaattggaagagtacttggccaagcaaggcagaccagcttctgatgctaaaatgttgagaattgacaagttggcttgcttgggttgctgttgcttctgtaccgttctttacatctgcaacgatgaatttttgaagaagaaccctgaaaaggtcagaaagttcttgaaagccatcaagaaggcaaccgactacgttctagccgaccctgtgaaggcttggaaagaatacatcgacttcaagcctcaattgaacaacgatctatcctacaagcaataccaaagatgttacgcttacttctcttcatctttgtacaatgttcaccgtgactggaagaaggttaccggttacggtaagagattagccatcttgccaccagactatgtctcgaactacactaatgaatacttgtcctggccagaaccagaagaggtttctgatcctttggaagctcaaagattgatggctattcatcaagaaaaatgcagacaggaaggtactttcaagagattggctcttccagcttaagcggccgcgagtcgtgagtaatcaagaggatgtcagaatgccatttgcctgagagatgcaggcttcatttttgatacttttttatttgtaacctatatagtataggattttttttgtcattttgtttcttctcgtacgagcttgctcctgatcagcctatctcgcagctgatgaatatcttgtggtaggggtttgggaaaatcattcgagtttgatgtttttcttggtatttcccactcctcttcagagtacagaagattaagtgagacgttcgtttgtgctccggaggatccttcagtaatgtcttgtttcttttgttgcagtggtgagccattttgacttcgtgaaagtttctttagaatagttgtttccagaggccaaacattccacccgtagtaaagtgcaagcgtaggaagaccaagactggcataaatcaggtataagtgtcgagcactggcaggtgatcttctgaaagtttctactagcagataagatccagtagtcatgcatatggcaacaatgtaccgtgtggatctaagaacgcgtcctactaaccttcgcattcgttggtccagtttgttgttatcgatcaacgtgacaaggttgtcgattccgcgtaagcatgcatacccaaggacgcctgttgcaattccaagtgagccagttccaacaatctttgtaatattagagcacttcattgtgttgcgcttgaaagtaaaatgcgaacaaattaagagataatctcgaaaccgcgacttcaaacgccaatatgatgtgcggcacacaataagcgttcatatccgctgggtgactttctcgctttaaaaaattatccgaaaaaattttctagagtgttgttactttatacttccggctcgtataatacgacaaggtgtaaggaggactaaaccatggctaaactcacctctgctgttccagtcctgactgctcgtgatgttgctggtgctgttgagttctggactgataggctcggtttctcccgtgacttcgtagaggacgactttgccggtgttgtacgtgacgacgttaccctgttcatctccgcagttcaggaccaggttgtgccagacaacactctggcatgggtatgggttcgtggtctggacgaactgtacgctgagtggtctgaggtcgtgtctaccaacttccgtgatgcatctggtccagctatgaccgagatcggtgaacagccctggggtcgtgagtttgcactgcgtgatccagctggtaactgcgtgcatttcgtcgcagaagagcaggactaacaattgacaccttacgattatttagagagtatttattagttttattgtatgtatacggatgttttattatctatttatgcccttatattctgtaactatccaaaagtcctatcttatcaagccagcaatctatgtccgcgaacgtcaactaaaaataagctttttatgctcttctctctttttttcccttcggtataattataccttgcatccacagattctcctgccaaattttgcataatcctttacaacatggctatatgggagcacttagcgccctccaaaacccatattgcctacgcatgtataggtgttttttccacaatattttctctgtgctctctttttattaaagagaagctctatatcggagaagcttctgtggccgttatattcggccttatcgtgggaccacattgcctgaattggtttgccccggaagattggggaaacttggatctgattaccttagctgcagaaaagggtaccactgagcgtcagaccccgtagaaaagatcaaaggatcttcttgagatcctttttttctgcgcgtaatctgctgcttgcaaacaaaaaaaccaccgctaccagcggtggtttgtttgccggatcaagagctaccaactctttttccgaaggtaactggcttcagcagagcgcagataccaaatactgttcttctagtgtagccgtagttaggccaccacttcaagaactctgtagcaccgcctacatacctcgctctgctaatcctgttaccagtggctgctgccagtggcgataagtcgtgtcttaccgggttggacccaagacgatagttaccggataaggcgcagcggtcgggctgaacggggggttcgtgcacacagcccagcttggagcgaacgacctacaccgaactgagatacctacagcgtgagctatgagaaagcgccacgcttcccgaagggagaaaggcggacaggtatccggtaagcggcagggtcggaacaggagagcgcacgagggagcttccagggggaaacgcctggtatctttatagtcctgtcgggtttcgccacctctgacttgagcgtcgatttttgtgatgctcgtcaggggggcggagcctatggaaaaacgccagcaacgcggcctttttacggttcctggccttttgctggccttttgctcacatgt

SEQ ID NO: 10 - DNA, 4756 bp, Artificial Sequence
  pGAPsec-Col45opt
  misc_feature (1)..(8): linearization site
  promoter (9)..(494): pGAP
  sig_peptide (495)..(761): MFalpha
  misc_feature (762)..(2309): Col45opt
  terminator (2313)..(2572): AOX TT
  promoter (2580)..(3137): PILV5
  promoter (3138)..(3201): PEM72
  misc_feature (3203)..(3577): ZeocinR
  terminator (3579)..(4054): TT
  rep_origin (4081)..(4754): pUC ORI
atttaaattttttgtagaaatgtcttggtgtcctcgtccaatcaggtagccatctctgaaatatctggctccgttgcaactccgaacgacctgctggcaacgtaaaattctccggggtaaaacttaaatgtggagtaatggaaccagaaacgtctcttcccttctctctccttccaccgcccgttaccgtccctaggaaattttactctgctggagagcttcttctacggcccccttgcagcaatgctcttcccagcattacgttgcgggtaaaacggaggtcgtgtacccgacctagcagcccagggatggaaaagtcccggccgtcgctggcaataatagcgggcggacgcatgtcatgagattattggaaaccaccagaatcgaatataaaaggcgaacacctttcccaattttggtttctcctgacccaaagactttaaatttaatttatttgtccctatttcaatcaattgaacaactatcaaaacacaatgagattcccatctattttcaccgctgtcttgttcgctgcctcctctgcattggctgcccctgttaacactaccactgaagacgagactgctcaaattccagctgaagcagttatcggttactctgaccttgagggtgatttcgacgtcgctgttttgcctttctctaactccactaacaacggtttgttgttcattaacaccactatcgcttccattgctgctaaggaagagggtgtctctctcgagaagagagaggccgaagctgagcgtggatttccaggcgaaaggggtgttcaaggcccacctggtcctgctggcccaagaggtgctaatggtgctcctggtaatgatggcgctaaaggtgacgccggtgctcccggtgcacccggttctcaaggtgcccctggcttgcaaggtatgccaggcgagcgtggtgctgctggattgcctggaccaaagggcgatagaggtgatgccggtccaaagggtgctgacggtgcaccaggtaaggacggtgtaagaggtttgactggacctattggccctccaggtccagccggtgcaccaggcgataagggtgaagctggaccttccggtccagctggccctactggtgctagaggtgccccaggtgatagaggcgagcctggtcctcctggacctgcaggctttgctggtcctcctggtgctgatggtcaacctggtgccaagggtgagccaggtgatgctggcgccaaaggtgatgcaggcccacctggacctgccggtcctgccggacctccaggtcctattggtaatgttggtgctcccggacctaaaggcgctagaggttcagccggtcctccaggcgctactggtttccctggtgctgcaggtagagttggtccaccaggtccatctggtaatgcaggaccaccaggtcctccaggtccagccggtaaagaaggttctaaaggtcctaggggtgaaactggtcccgcaggtaggcccggtgaagtaggccctccaggtcctcctggaccagctggcgaaaaaggtgctcctggcgcagatggtcctgccggcgctcctggaactccaggacctcagggtattgctggacaaagaggtgttgttggtctgccaggtcaacgtggtgaaagaggctttccaggactgcctggtccatcaggcgagccaggtaagcaaggaccatccggtgcttcaggcgaaagaggcccaccaggaccaatgggtccacctggtttagcaggacctccaggcgaatctggtagagaaggcgcaccaggcgctgaaggttctccaggtagagatggaagtcctggcgctaagggcgatcgtggcgaaactggccccgctggacctccaggcgctccaggtgctcccggcgctccaggaccagtcggtccagccggcaaatctggtgatagaggtgaaacaggcccagctggcccagccggaccaatcggtcctgttggtgctaggggtcccgctggtcctcaaggaccaaggggtgacaagggtgaaaccggtgaacagggtgatcgtggtattaagggacaccgtggattttccggattgcaaggacctcctggtcctccaggatctcccggtgaacaaggaccttctggtgcatctggacccgcaggacccaggggtccaccaggatctgctggaagtccaggtaaggatggtttgaacggtttgccaggaccaatcggccctcctggaccaagaggtagaactggtgatgccggaccagccggtccaccaggaccacctggacctccaggacctcctggtcctccttcttaatcaagaggatgtcagaatgccatttgcctgagagatgcaggcttcatttttgatacttttttatttgtaacctatatagtataggattttttttgtcattttgtttcttctcgtacgagcttgctcctgatcagcctatctcgcagctgatgaatatcttgtggtaggggtttgggaaaatcattcgagtttgatgtttttcttggtatttcccactcctcttcagagtacagaagattaagtgagacgttcgtttgtgctccggaggatccttcagtaatgtcttgtttcttttgttgcagtggtgagccattttgacttcgtgaaagtttctttagaatagttgtttccagaggccaaacattccacccgtagtaaagtgcaagcgtaggaagaccaagactggcataaatcaggtataagtgtcgagcactggcaggtgatcttctgaaagtttctactagcagataagatccagtagtcatgcatatggcaacaatgtaccgtgtggatctaagaacgcgtcctactaaccttcgcattcgttggtccagtttgttgttatcgatcaacgtgacaaggttgtcgattccgcgtaagcatgcatacccaaggacgcctgttgcaattccaagtgagccagttccaacaatctttgtaatattagagcacttcattgtgttgcgcttgaaagtaaaatgcgaacaaattaagagataatctcgaaaccgcgacttcaaacgccaatatgatgtgcggcacacaataagcgttcatatccgctgggtgactttctcgctttaaaaaattatccgaaaaaattttctagagtgttgttactttatacttccggctcgtataatacgacaaggtgtaaggaggactaaaccatggctaaactcacctctgctgttccagtcctgactgctcgtgatgttgctggtgctgttgagttctggactgataggctcggtttctcccgtgacttcgtagaggacgactttgccggtgttgtacgtgacgacgttaccctgttcatctccgcagttcaggaccaggttgtgccagacaacactctggcatgggtatgggttcgtggtctggacgaactgtacgctgagtggtctgaggtcgtgtctaccaacttccgtgatgcatctggtccagctatgaccgagatcggtgaacagccctggggtcgtgagtttgcactgcgtgatccagctggtaactgcgtgcatttcgtcgcagaagagcaggactaacaattgacaccttacgattatttagagagtatttattagttttattgtatgtatacggatgttttattatctatttatgcccttatattctgtaactatccaaaagtcctatcttatcaagccagcaatctatgtccgcgaacgtcaactaaaaataagctttttatgctcttctctctttttttcccttcggtataattataccttgcatccacagattctcctgccaaattttgcataatcctttacaacatggctatatgggagcacttagcgccctccaaaacccatattgcctacgcatgtataggtgttttttccacaatattttctctgtgctctctttttattaaagagaagctctatatcggagaagcttctgtggccgttatattcggccttatcgtgggaccacattgcctgaattggtttgccccggaagattggggaaacttggatctgattaccttagctgcagaaaagggtaccactgagcgtcagaccccgtagaaaagatcaaaggatcttcttgagatcctttttttctgcgcgtaatctgctgcttgcaaacaaaaaaaccaccgctaccagcggtggtttgtttgccggatcaagagctaccaactctttttccgaaggtaactggcttcagcagagcgcagataccaaatactgttcttctagtgtagccgtagttaggccaccacttcaagaactctgtagcaccgcctacatacctcgctctgctaatcctgttaccagtggctgctgccagtggcgataagtcgtgtcttaccgggttggacccaagacgatagttaccggataaggcgcagcggtcgggctgaacggggggttcgtgcacacagcccagcttggagcgaacgacctacaccgaactgagatacctacagcgtgagctatgagaaagcgccacgcttcccgaagggagaaaggcggacaggtatccggtaagcggcagggtcggaacaggagagcgcacgagggagcttccagggggaaacgcctggtatctttatagtcctgtcgggtttcgccacctctgacttgagcgtcgatttttgtgatgctcgtcaggggggcggagcctatggaaaaacgccagcaacgcggcctttttacggttcctggccttttgctggccttttgctcacatgt

SEQ ID NO: 11 - DNA, 4034 bp, Artificial Sequence
  pBSY3S1K
  misc_feature (1)..(8): linearization site
  promoter (9)..(508): PDC
  sig_peptide (509)..(733): Dalpha
  misc_feature (734)..(1166): Stuffer SapI Cloning
  terminator (1175)..(1434): AOX1TT
  promoter (1435)..(1992): PILV5
  promoter (1993)..(2056): PEM72
  misc_feature (2058)..(2867): kanMX6
  terminator (2868)..(3344): AODTT
  rep_origin (3359)..(4031): pUC ORI
atttaaattaatcgaactccgaatgcggttctcctgtaaccttaattgtagcatagatcacttaaataaactcatggcctgacatctgtacacgttcttattggtcttttagcaatcttgaagtctttctattgttccggtcggcattacctaataaattcgaatcgagattgctagtacctgatatcatatgaagtaatcatcacatgcaagttccatgataccctctactaatggaattgaacaaagtttaagcttctcgcacgagaccgaatccatactatgcacccctcaaagttgggattagtcaggaaagctgagcaattaacttccctcgattggcctggacttttcgcttagcctgccgcaatcggtaagtttcattatcccagcggggtgatagcctctgttgctcatcaggccaaaatcatatataagctgtagacccagcacttcaattacttgaaattcaccataacacttgctctagtcaagacttacaattaaaatgagattcccatctattttcaccgctgtcttgttcgctgcctcctctgcattggctgcccctgttaacactaccactgaagacgagactgctcaaattccagctgaagcagttatcggttactctgaccttgagggtgatttcgacgtcgctgttttgcctttctctgcttccattgctgctaaggaagagggtgtctctctcgagaagagagaggccgaagctagaagagcgaattcggcgcgccggtaagatccaaatcgatgaattgaccaagcactacggtatgaagccagaagactacactgctgtcagatgtggtatgaatgtcgccaagtacatcatcgaagataagattgatgctggtattggtatcgaatgtatgcaacaagtcgaattggaagagtacttggccaagcaaggcagaccagcttctgatgctaaaatgttgagaattgacaagttggcttgcttgggttgctgttgtttctgtaccgttctttacatctgcaacgatgaatttttgaagaaaaaccctgaaaaggtcagaaagttcttgaaagccatcaagaaggcaaccgactacgttctagccgaccctgtgaaggcttggaaagaatacatcgacttcaagcctcaattgaacagctcttcataagcggccgctcaagaggatgtcagaatgccatttgcctgagagatgcaggcttcatttttgatacttttttatttgtaacctatatagtataggattttttttgtcattttgtttcttctcgtacgagcttgctcctgatcagcctatctcgcagcagatgaatatcttgtggtaggggtttgggaaaatcattcgagtttgatgtttttcttggtatttcccactcctcttcagagtacagaagattaagtgagaccttcgtttgtgcgatccttcagtaatgtcttgtttcttttgttgcagtggtgagccattttgacttcgtgaaagtttctttagaatagttgtttccagaggccaaacattccacccgtagtaaagtgcaagcgtaggaagaccaagactggcataaatcaggtataagtgtcgagcactggcaggtgatcttctgaaagtttctactagcagataagatccagtagtcatgcatatggcaacaatgtaccgtgtggatctaagaacgcgtcctactaaccttcgcattcgttggtccagtttgttgttatcgatcaacgtgacaaggttgtcgattccgcgtaagcatgcatacccaaggacgcctgttgcaattccaagtgagccagttccaacaatctttgtaatattagagcacttcattgtgttgcgcttgaaagtaaaatgcgaacaaattaagagataatctcgaaaccgcgacttcaaacgccaatatgatgtgcggcacacaataagcgttcatatccgctgggtgactttctcgctttaaaaaattatccgaaaaaattttctagagtgttgacactttatacttccggctcgtataatacgacaaggtgtaaggaggactaaaccatgggtaaggaaaagactcacgtttcgaggccgcgattaaattccaacatggatgctgatttatatgggtataaatgggctcgcgataatgtcgggcaatcaggtgcgacaatctatcgattgtatgggaagcccgatgcgccagagttgtttctgaaacatggcaaaggtagcgttgccaatgatgttacagatgagatggtcagactaaactggctgacggaatttatgcctcttccgaccatcaagcattttatccgtactcctgatgatgcatggttactcaccactgcgatccccggcaaaacagcattccaggtattagaagaatatcctgattcaggtgaaaatattgttgatgcgctggcagtgttcctgcgccggttgcattcgattcctgtttgtaattgtccttttaacagcgatcgcgtatttcgtctcgctcaggcgcaatcacgaatgaataacggtttggttgatgcgagtgattttgatgacgagcgtaatggctggcctgttgaacaagtctggaaagaaatgcataagcttttgccattctcaccggattcagtcgtcactcatggtgatttctcacttgataaccttatttttgacgaggggaaattaataggttgtattgatgttggacgagtcggaatcgcagaccgataccaggatcttgccatcctatggaactgcctcggtgagttttctccttcattacagaaacggctttttcaaaaatatggtattgataatcctgatatgaataaattgcagtttcatttgatgctcgatgagtttttctaaaattgacaccttacgattatttagagagtatttattagttttattgtatgtatacggatgttttattatctatttatgcccttatattctgtaactatccaaaagtcctatcttatcaagccagcaatctatgtccgcgaacgtcaactaaaaataagctttttatcctcttctctctttttttcccttcggtataattataccttgcatccacagattctcctgccaaattttgcataatcctttacaacatggctatatgggagcacttagcgccctccaaaacccatattgcctacgcatgtataggtgttttttccacaatattttctctgtgctctctttttattaaagagaagctctatatcggagaagcttctgtggccgttatattcggccttatcgtgggaccacattgcctgaattggtttgccccggaagattggggaaacttggatctgattaccttagctgcagactgagcgtcagaccccgtagaaaagatcaaaggatcttcttgagatcctttttttctgcgcgtaatctgctgcttgcaaacaaaaaaaccaccgctaccagcggtggtttgtttgccggatcaagagctaccaactctttttccgaaggtaactggcttcagcagagcgcagataccaaatactgttcttctagtgtagccgtagttaggccaccacttcaagaactctgtagcaccgcctacatacctcgctctgctaatcctgttaccagtggctgctgccagtggcgataagtcgtgtcttaccgggttggactcaagacgatagttaccggataaggcgcagcggtcgggctgaacggggggttcgtgcacacagcccagcttggagcgaacgacctacaccgaactgagatacctacagcgtgagctatgagaaagcgccacgcttcccgaagggagaaaggcggacaggtatccggtaagcggcagggtcggaacaggagagcgcacgagggagcttccagggggaaacgcctggtatctttatagtcctgtcgggtttcgccacctctgacttgagcgtcgatttttgtgatgctcgtcaggggggcggagcctatggaaaaacgccagcaacgcggcctttttacggttcctggccttttgctggccttttgctcacatgt

SEQ ID NO: 12 - DNA, 4762 bp, Artificial Sequence
  pCATsec-Col45opt
  promoter (1)..(500): pCAT
  sig_peptide (501)..(557): preMFalpha
  sig_peptide (558)..(767): proMFalpha
  misc_feature (768)..(2315): Col45opt
  terminator (2319)..(2578): AOX TT
  promoter (2586)..(3143): PILV5
  promoter (3144)..(3207): PEM72
  misc_feature (3209)..(3583): ZeocinR
  terminator (3585)..(4060): TT
  rep_origin (4087)..(4760): pUC ori
taatcgaactccgaatgcggttctcctgtaaccttaattgtagcatagatcacttaaataaactcatggcctgacatctgtacacgttcttattggtcttttagcaatcttgaagtctttctattgttccggtcggcattacctaataaattcgaatcgagattgctagtacctgatatcatatgaagtaatcatcacatgcaagttccatgataccctctactaatggaattgaacaaagtttaagcttctcgcacgagaccgaatccatactatgcacccctcaaagttgggattagtcaggaaagctgagcaattaacttccctcgattggcctggacttttcgcttagcctgccgcaatcggtaagtttcattatcccagcggggtgatagcctctgttgctcatcaggccaaaatcatatataagctgtagacccagcacttcaattacttgaaattcaccataacacttgctctagtcaagacttacaattaaaatgagattcccatctattttcaccgctgtcttgttcgctgcctcctctgcattggctgcccctgttaacactaccactgaagacgagactgctcaaattccagctgaagcagttatcggttactctgaccttgagggtgatttcgacgtcgctgttttgcctttctctaactccactaacaacggtttgttgttcattaacaccactatcgcttccattgctgctaaggaagagggtgtctctctcgagaagagagaggccgaagctgagcgtggatttccaggcgaaaggggtgttcaaggcccacctggtcctgctggcccaagaggtgctaatggtgctcctggtaatgatggcgctaaaggtgacgccggtgctcccggtgcacccggttctcaaggtgcccctggcttgcaaggtatgccaggcgagcgtggtgctgctggattgcctggaccaaagggcgatagaggtgatgccggtccaaagggtgctgacggtgcaccaggtaaggacggtgtaagaggtttgactggacctattggccctccaggtccagccggtgcaccaggcgataagggtgaagctggaccttccggtccagctggccctactggtgctagaggtgccccaggtgatagaggcgagcctggtcctcctggacctgcaggctttgctggtcctcctggtgctgatggtcaacctggtgccaagggtgagccaggtgatgctggcgccaaaggtgatgcaggcccacctggacctgccggtcctgccggacctccaggtcctattggtaatgttggtgctcccggacctaaaggcgctagaggttcagccggtcctccaggcgctactggtttccctggtgctgcaggtagagttggtccaccaggtccatctggtaatgcaggaccaccaggtcctccaggtccagccggtaaagaaggttctaaaggtcctaggggtgaaactggtcccgcaggtaggcccggtgaagtaggccctccaggtcctcctggaccagctggcgaaaaaggtgctcctggcgcagatggtcctgccggcgctcctggaactccaggacctcagggtattgctggacaaagaggtgttgttggtctgccaggtcaacgtggtgaaagaggctttccaggactgcctggtccatcaggcgagccaggtaagcaaggaccatccggtgcttcaggcgaaagaggcccaccaggaccaatgggtccacctggtttagcaggacctccaggcgaatctggtagagaaggcgcaccaggcgctgaaggttctccaggtagagatggaagtcctggcgctaagggcgatcgtggcgaaactggccccgctggacctccaggcgctccaggtgctcccggcgctccaggaccagtcggtccagccggcaaatctggtgatagaggtgaaacaggcccagctggcccagccggaccaatcggtcctgttggtgctaggggtcccgctggtcctcaaggaccaaggggtgacaagggtgaaaccggtgaacagggtgatcgtggtattaagggacaccgtggattttccggattgcaaggacctcctggtcctccaggatctcccggtgaacaaggaccttctggtgcatctggacccgcaggacccaggggtccaccaggatctgctggaagtccaggtaaggatggtttgaacggtttgccaggaccaatcggccctcctggaccaagaggtagaactggtgatgccggaccagccggtccaccaggaccacctggacctccaggacctcctggtcctccttcttaatcaagaggatgtcagaatgccatttgcctgagagatgcaggcttcatttttgatacttttttatttgtaacctatatagtataggattttttttgtcattttgtttcttctcgtacgagcttgctcctgatcagcctatctcgcagctgatgaatatcttgtggtaggggtttgggaaaatcattcgagtttgatgtttttcttggtatttcccactcctcttcagagtacagaagattaagtgagacgttcgtttgtgctccggaggatccttcagtaatgtcttgtttcttttgttgcagtggtgagccattttgacttcgtgaaagtttctttagaatagttgtttccagaggccaaacattccacccgtagtaaagtgcaagcgtaggaagaccaagactggcataaatcaggtataagtgtcgagcactggcaggtgatcttctgaaagtttctactagcagataagatccagtagtcatgcatatggcaacaatgtaccgtgtggatctaagaacgcgtcctactaaccttcgcattcgttggtccagtttgttgttatcgatcaacgtgacaaggttgtcgattccgcgtaagcatgcatacccaaggacgcctgttgcaattccaagtgagccagttccaacaatctttgtaatattagagcacttcattgtgttgcgcttgaaagtaaaatgcgaacaaattaagagataatctcgaaaccgcgacttcaaacgccaatatgatgtgcggcacacaataagcgttcatatccgctgggtgactttctcgctttaaaaaattatccgaaaaaattttctagagtgttgttactttatacttccggctcgtataatacgacaaggtgtaaggaggactaaaccatggctaaactcacctctgctgttccagtcctgactgctcgtgatgttgctggtgctgttgagttctggactgataggctcggtttctcccgtgacttcgtagaggacgactttgccggtgttgtacgtgacgacgttaccctgttcatctccgcagttcaggaccaggttgtgccagacaacactctggcatgggtatgggttcgtggtctggacgaactgtacgctgagtggtctgaggtcgtgtctaccaacttccgtgatgcatctggtccagctatgaccgagatcggtgaacagccctggggtcgtgagtttgcactgcgtgatccagctggtaactgcgtgcatttcgtcgcagaagagcaggactaacaattgacaccttacgattatttagagagtatttattagttttattgtatgtatacggatgttttattatctatttatgcccttatattctgtaactatccaaaagtcctatcttatcaagccagcaatctatgtccgcgaacgtcaactaaaaataagctttttatgctcttctctctttttttcccttcggtataattataccttgcatccacagattctcctgccaaattttgcataatcctttacaacatggctatatgggagcacttagcgccctccaaaacccatattgcctacgcatgtataggtgttttttccacaatattttctctgtgctctctttttattaaagagaagctctatatcggagaagcttctgtggccgttatattcggccttatcgtgggaccacattgcctgaattggtttgccccggaagattggggaaacttggatctgattaccttagctgcagaaaagggtaccactgagcgtcagaccccgtagaaaagatcaaaggatcttcttgagatcctttttttctgcgcgtaatctgctgcttgcaaacaaaaaaaccaccgctaccagcggtggtttgtttgccggatcaagagctaccaactctttttccgaaggtaactggcttcagcagagcgcagataccaaatactgttcttctagtgtagccgtagttaggccaccacttcaagaactctgtagcaccgcctacatacctcgctctgctaatcctgttaccagtggctgctgccagtggcgataagtcgtgtcttaccgggttggacccaagacgatagttaccggataaggcgcagcggtcgggctgaacggggggttcgtgcacacagcccagcttggagcgaacgacctacaccgaactgagatacctacagcgtgagctatgagaaagcgccacgcttcccgaagggagaaaggcggacaggtatccggtaagcggcagggtcggaacaggagagcgcacgagggagcttccagggggaaacgcctggtatctttatagtcctgtcgggtttcgccacctctgacttgagcgtcgatttttgtgatgctcgtcaggggggcggagcctatggaaaaacgccagcaacgcggcctttttacggttcctggccttttgctggccttttgctcacatgt

SEQ ID NO: 13 - DNA, 1191 bp, Pichia pastoris
atgaaagttgtctggttagcatgtttcataatactggcagctatatggtataaagactaccaaagtttaagaggattcatggacgacagagtgtcgaagaccttgccaattaattttaacgcactaaagttatctaccaattcttatatacccgtggatgagcaccttataaagcctaacagagaaccgaacccaaaatttgttaaagaaaatgctactttgctgatgttatgccgaaattgggaactagaagaagtactgcaatcaatgagatcactcgaagataggttcaatggtaggtatcagtatacttggacattcttgaatgatgtgccctttgagaaacagttcatacaggaaacaactttgatggcctcggggaaaactcaatatgcgttaatttctagcacagattggaatagaccttcttttataaacgaaacgaggttcgaacagaatttaatccaatctgagaaggatgatatcatctacggtggaagtccatcttatcgaaatatgtgccgtttcaattcaggattcttttacaaacaaaagatactcgaccaatatgattattattttagagtggaacccggagtggagtacttttgtgatttagaagaggatccattcagatatatgagacttcacgataaaaagtatgggtttgtcatttcactttacgagtatgaaaacaccattccaacgttatggcagaccgttgaaaaattcatagaaaatcatccagagtacatccacccaaacaactcctacgaatttttaactgacaaggaagttgttggccctttaggcttagttgcattaactgaacagacttataatctgtgccatttttggtctaattttgaaattggagatttgaacttttttagaagtgaaaagtacgaggcttttttccagtttctggatcaggctggaggattttattatgaaagatggggagatgccccagtgcattcgatagcagttggcattttgttagataagagacagatacaccattttgagaatattggttattaccatcttccattcagcacatgtccccagtcatattggtcatacaagtgcaatagatgcatttgcaagcggaatgaatccatcgatttagttccacatagttgtcttagcaaatggtggaaatatggaggtaaaacattcctccaatag

SEQ ID NO: 14 - protein, 396 aa, Pichia pastoris
MKVVWLACFIILAAIWYKDYQSLRGFMDDRVSKTLPINFNALKLSTNSYIPVDEHLIKPNREPNPKFVKENATLLMLCRNWELEEVLQSMRSLEDRFNGRYQYTWTFLNDVPFEKQFIQETTLMASGKTQYALISSTDWNRPSFINETRFEQNLIQSEKDDIIYGGSPSYRNMCRFNSGFFYKQKILDQYDYYFRVEPGVEYFCDLEEDPFRYMRLHDKKYGFVISLYEYENTIPTLWQTVEKFIENHPEYIHPNNSYEFLTDKEVVGPLGLVALTEQTYNLCHFWSNFEIGDLNFFRSEKYEAFFQFLDQAGGFYYERWGDAPVHSIAVGILLDKRQIHHFENIGYYHLPFSTCPQSYWSYKCNRCICKRNESIDLVPHSCLSKWWKYGGKTFLQ

SEQ ID NO: 15 - DNA, 1167 bp, Artificial Sequence
  truncated yur1
atgaaagttgtctggttagcatgtttcataatactggcagctatatggtataaagactaccaaagtttaagaggattcatggacgacagagtgtcgaagaccttgccaattaattttaacgcactaaagttatctaccaattcttatatacccgtggatgagcaccttataaagcctaacagagaaccgaacccaaaatttgttaaagaaaatgctactttgctgatgttatgccgaaattgggaactagaagaagtactgcaatcaatgagatcactcgaagataggttcaatggtaggtatcagtatacttggacattcttgaatgatgtgccctttgagaaacagttcatacaggaaacaactttgatggcctcggggaaaactcaatatgcgttaatttctagcacagattggaatagaccttcttttataaacgaaacgaggttcgaacagaatttaatccaatctgagaaggatgatatcatctacggtggaagtccatcttatcgaaatatgtgccgtttcaattcaggattcttttacaaacaaaagatactcgaccaatatgattattattttagagtggaacccggagtggagtacttttgtgatttagaagaggatccattcagatatatgagacttcacgataaaaagtatgggtttgtcatttcactttacgagtatgaaaacaccattccaacgttatggcagaccgttgaaaaattcatagaaaatcatccagagtacatccacccaaacaactcctacgaatttttaactgacaaggaagttgttggccctttaggcttagttgcattaactgaacagacttataatctgtgccatttttggtctaattttgaaattggagatttgaacttttttagaagtgaaaagtacgaggcttttttccagtttctggatcaggctggaggattttattatgaaagatggggagatgccccagtgcattcgatagcagttggcattttgttagataagagacagatacaccattttgagaatattggttattaccatcttccattcagcacatgtccccagtcatattggtcatacaagtgcaatagatgcatttgcaagcggaatgaatccatcgatttagttccacatagttgtcttagcaatcgagattgctag

SEQ ID NO: 16 - protein, 388 aa, Artificial Sequence
  truncated Yur1
MKVVWLACFIILAAIWYKDYQSLRGFMDDRVSKTLPINFNALKLSTNSYIPVDEHLIKPNREPNPKFVKENATLLMLCRNWELEEVLQSMRSLEDRFNGRYQYTWTFLNDVPFEKQFIQETTLMASGKTQYALISSTDWNRPSFINETRFEQNLIQSEKDDIIYGGSPSYRNMCRFNSGFFYKQKILDQYDYYFRVEPGVEYFCDLEEDPFRYMRLHDKKYGFVISLYEYENTIPTLWQTVEKFIENHPEYIHPNNSYEFLTDKEVVGPLGLVALTEQTYNLCHFWSNFEIGDLNFFRSEKYEAFFQFLDQAGGFYYERWGDAPVHSIAVGILLDKRQIHHFENIGYYHLPFSTCPQSYWSYKCNRCICKRNESIDLVPHSCLSNRDC

SEQ ID NO: 17 - DNA, 5953 bp, Artificial Sequence
  pCATsec-Col45yur1
  promoter (1)..(500): pCAT
  sig_peptide (501)..(767): MFalpha
  sig_peptide (501)..(557): preMFalpha
  misc_feature (768)..(2315): Col45opt
  terminator (2319)..(2578): TT
  promoter (2586)..(3143): PILV5
  promoter (3144)..(3207): PEM72
  misc_feature (3209)..(3583): ZeocinR
  terminator (3585)..(4060): TT
  rep_origin (4087)..(4760): pUC ori
  misc_feature (4763)..(5953): yur1
taatcgaactccgaatgcggttctcctgtaaccttaattgtagcatagatcacttaaataaactcatggcctgacatctgtacacgttcttattggtcttttagcaatcttgaagtctttctattgttccggtcggcattacctaataaattcgaatcgagattgctagtacctgatatcatatgaagtaatcatcacatgcaagttccatgataccctctactaatggaattgaacaaagtttaagcttctcgcacgagaccgaatccatactatgcacccctcaaagttgggattagtcaggaaagctgagcaattaacttccctcgattggcctggacttttcgcttagcctgccgcaatcggtaagtttcattatcccagcggggtgatagcctctgttgctcatcaggccaaaatcatatataagctgtagacccagcacttcaattacttgaaattcaccataacacttgctctagtcaagacttacaattaaaatgagattcccatctattttcaccgctgtcttgttcgctgcctcctctgcattggctgcccctgttaacactaccactgaagacgagactgctcaaattccagctgaagcagttatcggttactctgaccttgagggtgatttcgacgtcgctgttttgcctttctctaactccactaacaacggtttgttgttcattaacaccactatcgcttccattgctgctaaggaagagggtgtctctctcgagaagagagaggccgaagctgagcgtggatttccaggcgaaaggggtgttcaaggcccacctggtcctgctggcccaagaggtgctaatggtgctcctggtaatgatggcgctaaaggtgacgccggtgctcccggtgcacccggttctcaaggtgcccctggcttgcaaggtatgccaggcgagcgtggtgctgctggattgcctggaccaaagggcgatagaggtgatgccggtccaaagggtgctgacggtgcaccaggtaaggacggtgtaagaggtttgactggacctattggccctccaggtccagccggtgcaccaggcgataagggtgaagctggaccttccggtccagctggccctactggtgctagaggtgccccaggtgatagaggcgagcctggtcctcctggacctgcaggctttgctggtcctcctggtgctgatggtcaacctggtgccaagggtgagccaggtgatgctggcgccaaaggtgatgcaggcccacctggacctgccggtcctgccggacctccaggtcctattggtaatgttggtgctcccggacctaaaggcgctagaggttcagccggtcctccaggcgctactggtttccctggtgctgcaggtagagttggtccaccaggtccatctggtaatgcaggaccaccaggtcctccaggtccagccggtaaagaaggttctaaaggtcctaggggtgaaactggtcccgcaggtaggcccggtgaagtaggccctccaggtcctcctggaccagctggcgaaaaaggtgctcctggcgcagatggtcctgccggcgctcctggaactccaggacctcagggtattgctggacaaagaggtgttgttggtctgccaggtcaacgtggtgaaagaggctttccaggactgcctggtccatcaggcgagccaggtaagcaaggaccatccggtgcttcaggcgaaagaggcccaccaggaccaatgggtccacctggtttagcaggacctccaggcgaatctggtagagaaggcgcaccaggcgctgaaggttctccaggtagagatggaagtcctggcgctaagggcgatcgtggcgaaactggccccgctggacctccaggcgctccaggtgctcccggcgctccaggaccagtcggtccagccggcaaatctggtgatagaggtgaaacaggcccagctggcccagccggaccaatcggtcctgttggtgctaggggtcccgctggtcctcaaggaccaaggggtgacaagggtgaaaccggtgaacagggtgatcgtggtattaagggacaccgtggattttccggattgcaaggacctcctggtcctccaggatctcccggtgaacaaggaccttctggtgcatctggacccgcaggacccaggggtccaccaggatctgctggaagtccaggtaaggatggtttgaacggtttgccaggaccaatcggccctcctggaccaagaggtagaactggtgatgccggaccagccggtccaccaggaccacctggacctccaggacctcctggtcctccttcttaatcaagaggatgtcagaatgccatttgcctgagagatgcaggcttcatttttgatacttttttatttgtaacctatatagtataggattttttttgtcattttgtttcttctcgtacgagcttgctcctgatcagcctatctcgcagctgatgaatatcttgtggtaggggtttgggaaaatcattcgagtttgatgtttttcttggtatttcccactcctcttcagagtacagaagattaagtgagacgttcgtttgtgctccggaggatccttcagtaatgtcttgtttcttttgttgcagtggtgagccattttgacttcgtgaaagtttctttagaatagttgtttccagaggccaaacattccacccgtagtaaagtgcaagcgtaggaagaccaagactggcataaatcaggtataagtgtcgagcactggcaggtgatcttctgaaagtttctactagcagataagatccagtagtcatgcatatggcaacaatgtaccgtgtggatctaagaacgcgtcctactaaccttcgcattcgttggtccagtttgttgttatcgatcaacgtgacaaggttgtcgattccgcgtaagcatgcatacccaaggacgcctgttgcaattccaagtgagccagttccaacaatctttgtaatattagagcacttcattgtgttgcgcttgaaagtaaaatgcgaacaaattaagagataatctcgaaaccgcgacttcaaacgccaatatgatgtgcggcacacaataagcgttcatatccgctgggtgactttctcgctttaaaaaattatccgaaaaaattttctagagtgttgttactttatacttccggctcgtataatacgacaaggtgtaaggaggactaaaccatggctaaactcacctctgctgttccagtcctgactgctcgtgatgttgctggtgctgttgagttctggactgataggctcggtttctcccgtgacttcgtagaggacgactttgccggtgttgtacgtgacgacgttaccctgttcatctccgcagttcaggaccaggttgtgccagacaacactctggcatgggtatgggttcgtggtctggacgaactgtacgctgagtggtctgaggtcgtgtctaccaacttccgtgatgcatctggtccagctatgaccgagatcggtgaacagccctggggtcgtgagtttgcactgcgtgatccagctggtaactgcgtgcatttcgtcgcagaagagcaggactaacaattgacaccttacgattatttagagagtatttattagttttattgtatgtatacggatgttttattatctatttatgcccttatattctgtaactatccaaaagtcctatcttatcaagccagcaatctatgtccgcgaacgtcaactaaaaataagctttttatgctcttctctctttttttcccttcggtataattataccttgcatccacagattctcctgccaaattttgcataatcctttacaacatggctatatgggagcacttagcgccctccaaaacccatattgcctacgcatgtataggtgttttttccacaatattttctctgtgctctctttttattaaagagaagctctatatcggagaagcttctgtggccgttatattcggccttatcgtgggaccacattgcctgaattggtttgccccggaagattggggaaacttggatctgattaccttagctgcagaaaagggtaccactgagcgtcagaccccgtagaaaagatcaaaggatcttcttgagatcctttttttctgcgcgtaatctgctgcttgcaaacaaaaaaaccaccgctaccagcggtggtttgtttgccggatcaagagctaccaactctttttccgaaggtaactggcttcagcagagcgcagataccaaatactgttcttctagtgtagccgtagttaggccaccacttcaagaactctgtagcaccgcctacatacctcgctctgctaatcctgttaccagtggctgctgccagtggcgataagtcgtgtcttaccgggttggacccaagacgatagttaccggataaggcgcagcggtcgggctgaacggggggttcgtgcacacagcccagcttggagcgaacgacctacaccgaactgagatacctacagcgtgagctatgagaaagcgccacgcttcccgaagggagaaaggcggacaggtatccggtaagcggcagggtcggaacaggagagcgcacgagggagcttccagggggaaacgcctggtatctttatagtcctgtcgggtttcgccacctctgacttgagcgtcgatttttgtgatgctcgtcaggggggcggagcctatggaaaaacgccagcaacgcggcctttttacggttcctggccttttgctggccttttgctcacatgtatgaaagttgtctggttagcatgtttcataatactggcagctatatggtataaagactaccaaagtttaagaggattcatggacgacagagtgtcgaagaccttgccaattaattttaacgcactaaagttatctaccaattcttatatacccgtggatgagcaccttataaagcctaacagagaaccgaacccaaaatttgttaaagaaaatgctactttgctgatgttatgccgaaattgggaactagaagaagtactgcaatcaatgagatcactcgaagataggttcaatggtaggtatcagtatacttggacattcttgaatgatgtgccctttgagaaacagttcatacaggaaacaactttgatggcctcggggaaaactcaatatgcgttaatttctagcacagattggaatagaccttcttttataaacgaaacgaggttcgaacagaatttaatccaatctgagaaggatgatatcatctacggtggaagtccatcttatcgaaatatgtgccgtttcaattcaggattcttttacaaacaaaagatactcgaccaatatgattattattttagagtggaacccggagtggagtacttttgtgatttagaagaggatccattcagatatatgagacttcacgataaaaagtatgggtttgtcatttcactttacgagtatgaaaacaccattccaacgttatggcagaccgttgaaaaattcatagaaaatcatccagagtacatccacccaaacaactcctacgaatttttaactgacaaggaagttgttggccctttaggcttagttgcattaactgaacagacttataatctgtgccatttttggtctaattttgaaattggagatttgaacttttttagaagtgaaaagtacgaggcttttttccagtttctggatcaggctggaggattttattatgaaagatggggagatgccccagtgcattcgatagcagttggcattttgttagataagagacagatacaccattttgagaatattggttattaccatcttccattcagcacatgtccccagtcatattggtcatacaagtgcaatagatgcatttgcaagcggaatgaatccatcgatttagttccacatagttgtcttagcaaatggtggaaatatggaggtaaaacattcctccaatag

SEQ ID NO: 18 - DNA, 4348 bp, Artificial Sequence
  pAOX_Mimi-int_3.0
  misc_feature (1)..(8): linearization site
  promoter (15)..(948): PAOX
  misc_feature (949)..(1014): Ost1
  misc_feature (1015)..(1713): P4H
  terminator (1714)..(1973): AOX1TT
  promoter (1975)..(2532): PILV5
  promoter (2533)..(2596): PEM72
  misc_feature (2598)..(3413): kanMX
  terminator (3414)..(3653): tAgTEF
  rep_origin (3673)..(4343): pUC
atttaaatagatctaacatccaaagacgaaaggttgaatgaaacctttttgccatccgacatccacaggtccattctcacacataagtgccaaacgcaacaggaggggatacactagcagcagaccgttgcaaacgcaggacctccactcctcttctcctcaacacccacttttgccatcgaaaaaccagcccagttattgggcttgattggagctcgctcattccaattccttctattaggctactaacaccatgactttattagcctgtctatcctggcccccctggcgaggttcatgtttgtttatttccgaatgcaacaagctccgcattacacccgaacatcactccagatgagggctttctgagtgtggggtcaaatagtttcatgttccccaaatggcccaaaactgacagtttaaacgctgtcttggaacctaatatgacaaaagcgtgatctcatccaagatgaactaagtttggttcgttgaaatgctaacggccagttggtcaaaaagaaacttccaaaagtcggcataccgtttgtcttgtttggtattgattgacgaatgctcaaaaataatctcattaatgcttagcgcagtctctctatcgcttctgaaccccggtgcacctgtgccgaaacgcaaatggggaaacacccgctttttggatgattatgcattgtctccacattgtatgcttccaagattctggtgggaatactgctgatagcctaacgttcatgatcaaaatttaactgttctaacccctacttgacagcaatatataaacagaaggaagctgccctgtcttaaacctttttttttatcatcattattagcttactttcataattgcgactggttccaattgacaagcttttgattttaacgacttttaacgacaacttgagaagatcaaaaaacaactaattattcgaaacgatgaggcaggtttggttctcttggattgtgggattgttcctatgttttttcaacgtgtcttctgctcatcatcaccaccatcacatggttctgtccaaatcctgtgtttcacacttccgaaatgtaggttctctaaacagtagagatgttaatcttaaagacgatttcagctatgccaatattgatgatccttacaataagccatttgtgcttaataacctgattaaccctactaagtgtcaagaaatcatgcaatttgcaaatggcaagttgtttgattcacaggttttgtctgggactgacaagaacattagaaactcgcaacaaatgtggattagcaagaacaatcctatggtaaagccaatctttgagaatatttgcagacagttcaatgttccctttgacaatgctgaagatttgcaagtcgttcgttatcttccaaaccagtactataacgaacaccatgactcgtgttgtgactcttcaaaacaatgcagtgagttcattgagagaggtggtcaaaggattttgacagtcttgatctacctaaacaatgagttcagtgatggacacacttactttccgaacttaaaccagaaattcaagcccaaaactggagatgcattagtcttttatccattggccaataactctaacaaatgccatccatactccttacatgctggtatgcctgtaacatctggagaaaagtggattgctaatttgtggtttagagaacgtaaattctcccatgatgaattgtaatcaagaggatgtcagaatgccatttgcctgagagatgcaggcttcatttttgatacttttttatttgtaacctatatagtataggattttttttgtcattttgtttcttctcgtacgagcttgctcctgatcagcctatctcgcagcagatgaatatcttgtggtaggggtttgggaaaatcattcgagtttgatgtttttcttggtatttcccactcctcttcagagtacagaagattaagtgagaccttcgtttgtgcggatccttcagtaatgtcttgtttcttttgttgcagtggtgagccattttgacttcgtgaaagtttctttagaatagttgtttccagaggccaaacattccacccgtagtaaagtgcaagcgtaggaagaccaagactggcataaatcaggtataagtgtcgagcactggcaggtgatcttctgaaagtttctactagcagataagatccagtagtcatgcatatggcaacaatgtaccgtgtggatctaagaacgcgtcctactaaccttcgcattcgttggtccagtttgttgttatcgatcaacgtgacaaggttgtcgattccgcgtaagcatgcatacccaaggacgcctgttgcaattccaagtgagccagttccaacaatctttgtaatattagagcacttcattgtgttgcgcttgaaagtaaaatgcgaacaaattaagagataatctcgaaaccgcgacttcaaacgccaatatgatgtgcggcacacaataagcgttcatatccgctgggtgactttctcgctttaaaaaattatccgaaaaaattttctagagtgttgttactttatacttccggctcgtataatacgacaaggtgtaaggaggactaaaccatgagccatattcaacgggaaacgtcttgctcgaggccgcgattaaattccaacatggatgctgatttatatgggtataaatgggctcgcgataatgtcgggcaatcaggtgcgacaatctatcgattgtatgggaagcccgatgcgccagagttgtttctgaaacatggcaaaggtagcgttgccaatgatgttacagatgagatggtcagactaaactggctgacggaatttatgcctcttccgaccatcaagcattttatccgtactcctgatgatgcatggttactcaccactgcgatccccggcaaaacagcattccaggtattagaagaatatcctgattcaggtgaaaatattgttgatgcgctggcagtgttcctgcgccggttgcattcgattcctgtttgtaattgtccttttaacagcgatcgcgtatttcgtctcgctcaggcgcaatcacgaatgaataacggtttggttgatgcgagtgattttgatgacgagcgtaatggctggcctgttgaacaagtctggaaagaaatgcataagcttttgccattctcaccggattcagtcgtcactcatggtgatttctcacttgataaccttatttttgacgaggggaaattaataggttgtattgatgttggacgagtcggaatcgcagaccgataccaggatcttgccatcctatggaactgcctcggtgagttttctccttcattacagaaacggctttttcaaaaatatggtattgataatcctgatatgaataaattgcagtttcatttgatgctcgatgagtttttctaatcagtactgacaataaaaagattcttgttttcaagaacttgtcatttgtatagtttttttatattgtagttgttctattttaatcaaatgttagcgtgatttatattttttttcgcctcgacatcatctgcccagatgcgaagttaagtgcgcagaaagtaatatcatgcgtcaatcgtatgtgaatgctggtcgctatactgctgtcgattcgatactaacgccgccatccagtgtcgagtaccactgagcgtcagaccccgtagaaaagatcaaaggatcttcttgagatcctttttttctgcgcgtaatctgctgcttgcaaacaaaaaaaccaccgctaccagcggtggtttgtttgccggatcaagagctaccaactctttttccgaaggtaactggcttcagcagagcgcagataccaaatactgttcttctagtgtagccgtagttaggccaccacttcaagaactctgtagcaccgcctacatacctcgctctgctaatcctgttaccagtggctgctgccagtggcgataagtcgtgtcttaccgggttggactcaagacgatagttaccggataaggcgcagcggtcgggctgaacggggggttcgtgcacacagcccagcttggagcgaacgacctacaccgaactgagatacctacagcgtgagctatgagaaagcgccacgcttcccgaagggagaaaggcggacaggtatccggtaagcggcagggtcggaacaggagagcgcacgagggagcttccagggggaaacgcctggtatctttatagtcctgtcgggtttcgccacctctgacttgagcgtcgatttttgtgatgctcgtcaggggggcggagcctatggaaaaacgccagcaacgcggcctttttacggttcctggccttttgctggccttttgctcacatgt

SEQ ID NO: 19 - DNA, 4561 bp, Artificial Sequence
  pAOX_Mimi-int_3.1
  misc_feature (1)..(8): linearization site
  promoter (15)..(948): PAOX
  misc_feature (949)..(1014): Ost1
  misc_feature (1015)..(1713): P4H
  terminator (1714)..(1973): AOX1TT
  promoter (1975)..(2532): PILV5
  promoter (2533)..(2596): PEM72
  misc_feature (2598)..(3626): HygR
  terminator (3627)..(3866): tAgTEF
  rep_origin (3886)..(4556): pUC
atttaaatagatctaacatccaaagacgaaaggttgaatgaaacctttttgccatccgacatccacaggtccattctcacacataagtgccaaacgcaacaggaggggatacactagcagcagaccgttgcaaacgcaggacctccactcctcttctcctcaacacccacttttgccatcgaaaaaccagcccagttattgggcttgattggagctcgctcattccaattccttctattaggctactaacaccatgactttattagcctgtctatcctggcccccctggcgaggttcatgtttgtttatttccgaatgcaacaagctccgcattacacccgaacatcactccagatgagggctttctgagtgtggggtcaaatagtttcatgttccccaaatggcccaaaactgacagtttaaacgctgtcttggaacctaatatgacaaaagcgtgatctcatccaagatgaactaagtttggttcgttgaaatgctaacggccagttggtcaaaaagaaacttccaaaagtcggcataccgtttgtcttgtttggtattgattgacgaatgctcaaaaataatctcattaatgcttagcgcagtctctctatcgcttctgaaccccggtgcacctgtgccgaaacgcaaatggggaaacacccgctttttggatgattatgcattgtctccacattgtatgcttccaagattctggtgggaatactgctgatagcctaacgttcatgatcaaaatttaactgttctaacccctacttgacagcaatatataaacagaaggaagctgccctgtcttaaacctttttttttatcatcattattagcttactttcataattgcgactggttccaattgacaagcttttgattttaacgacttttaacgacaacttgagaagatcaaaaaacaactaattattcgaaacgatgaggcaggtttggttctcttggattgtgggattgttcctatgttttttcaacgtgtcttctgctcatcatcaccaccatcacatggttctgtccaaatcctgtgtttcacacttccgaaatgtaggttctctaaacagtagagatgttaatcttaaagacgatttcagctatgccaatattgatgatccttacaataagccatttgtgcttaataacctgattaaccctactaagtgtcaagaaatcatgcaatttgcaaatggcaagttgtttgattcacaggttttgtctgggactgacaagaacattagaaactcgcaacaaatgtggattagcaagaacaatcctatggtaaagccaatctttgagaatatttgcagacagttcaatgttccctttgacaatgctgaagatttgcaagtcgttcgttatcttccaaaccagtactataacgaacaccatgactcgtgttgtgactcttcaaaacaatgcagtgagttcattgagagaggtggtcaaaggattttgacagtcttgatctacctaaacaatgagttcagtgatggacacacttactttccgaacttaaaccagaaattcaagcccaaaactggagatgcattagtcttttatccattggccaataactctaacaaatgccatccatactccttacatgctggtatgcctgtaacatctggagaaaagtggattgctaatttgtggtttagagaacgtaaattctcccatgatgaattgtaatcaagaggatgtcagaatgccatttgcctgagagatgcaggcttcatttttgatacttttttatttgtaacctatatagtataggattttttttgtcattttgtttcttctcgtacgagcttgctcctgatcagcctatctcgcagcagatgaatatcttgtggtaggggtttgggaaaatcattcgagtttgatgtttttcttggtatttcccactcctcttcagagtacagaagattaagtgagaccttcgtttgtgcggatccttcagtaatgtcttgtttcttttgttgcagtggtgagccattttgacttcgtgaaagtttctttagaatagttgtttccagaggccaaacattccacccgtagtaaagtgcaagcgtaggaagaccaagactggcataaatcaggtataagtgtcgagcactggcaggtgatcttctgaaagtttctactagcagataagatccagtagtcatgcatatggcaacaatgtaccgtgtggatctaagaacgcgtcctactaaccttcgcattcgttggtccagtttgttgttatcgatcaacgtgacaaggttgtcgattccgcgtaagcatgcatacccaaggacgcctgttgcaattccaagtgagccagttccaacaatctttgtaatattagagcacttcattgtgttgcgcttgaaagtaaaatgcgaacaaattaagagataatctcgaaaccgcgacttcaaacgccaatatgatgtgcggcacacaataagcgttcatatccgctgggtgactttctcgctttaaaaaattatccgaaaaaattttctagagtgttgttactttatacttccggctcgtataatacgacaaggtgtaaggaggactaaaccatgggtaaaaagcctgaactcaccgcgacgtctgtcgagaagtttctgatcgaaaagttcgacagcgtctccgacctgatgcagctctcggagggcgaagaatctcgtgctttcagcttcgatgtaggagggcgtggatatgtcctgcgggtaaatagctgcgccgatggtttctacaaagatcgttatgtttatcggcactttgcatcggccgcgctcccgattccggaagtgcttgacattggggaattcagcgagagcctgacctattgcatctcccgccgtgcacagggtgtcacgttgcaagacctgcctgaaaccgaactgcccgctgttctgcagccggtcgcggaggcaatggatgcgatcgctgcggccgatcttagccagacgagcgggttcggcccattcggaccgcaaggaatcggtcaatacactacatggcgtgatttcatatgcgcgattgctgatccccatgtgtatcactggcaaactgtgatggacgacaccgtcagtgcgtccgtcgcgcaggctctcgatgagctgatgctttgggccgaggactgccccgaagtccggcacctcgtgcacgcggatttcggctccaacaatgtcctgacggacaatggccgcataacagcggtcattgactggagcgaggcgatgttcggggattcccaatacgaggtcgccaacatcttcttctggaggccgtggttggcttgtatggagcagcagacgcgctacttcgagcggaggcatccggagcttgcaggatcgccgcggctccgggcgtatatgctccgcattggtcttgaccaactctatcagagcttggttgacggcaatttcgatgatgcagcttgggcgcagggtcgatgcgacgcaatcgtccgatccggagccgggactgtcgggcgtacacaaatcgcccgcagaagcgcggccgtctggaccgatggctgtgtagaagtactcgccgatagtggaaaccgacgccccagcactcgtccgagggcaaaggaataatcagtactgacaataaaaagattcttgttttcaagaacttgtcatttgtatagtttttttatattgtagttgttctattttaatcaaatgttagcgtgatttatattttttttcgcctcgacatcatctgcccagatgcgaagttaagtgcgcagaaagtaatatcatgcgtcaatcgtatgtgaatgctggtcgctatactgctgtcgattcgatactaacgccgccatccagtgtcgagtaccactgagcgtcagaccccgtagaaaagatcaaaggatcttcttgagatcctttttttctgcgcgtaatctgctgcttgcaaacaaaaaaaccaccgctaccagcggtggtttgtttgccggatcaagagctaccaactctttttccgaaggtaactggcttcagcagagcgcagataccaaatactgttcttctagtgtagccgtagttaggccaccacttcaagaactctgtagcaccgcctacatacctcgctctgctaatcctgttaccagtggctgctgccagtggcgataagtcgtgtcttaccgggttggactcaagacgatagttaccggataaggcgcagcggtcgggctgaacggggggttcgtgcacacagcccagcttggagcgaacgacctacaccgaactgagatacctacagcgtgagctatgagaaagcgccacgcttcccgaagggagaaaggcggacaggtatccggtaagcggcagggtcggaacaggagagcgcacgagggagcttccagggggaaacgcctggtatctttatagtcctgtcgggtttcgccacctctgacttgagcgtcgatttttgtgatgctcgtcaggggggcggagcctatggaaaaacgccagcaacgcggcctttttacggttcctggccttttgctggccttttgctcacatgt

SEQ ID NO: 20 - DNA, 267 bp, Artificial Sequence
  artificial MF alpha
atgagattcccatctattttcaccgctgtcttgttcgctgcctcctctgcattggctgcccctgttaacactaccactgaagacgagactgctcaaattccagctgaagcagttatcggttactctgaccttgagggtgatttcgacgtcgctgttttgcctttctctaactccactaacaacggtttgttgttcattaacaccactatcgcttccattgctgctaaggaagagggtgtctctctcgagaagagagaggccgaagct

SEQ ID NO: 21 - protein, 89 aa, Artificial Sequence
  artificial MF alpha
MRFPSIFTAVLFAASSALAAPVNTTTEDETAQIPAEAVIGYSDLEGDFDVAVLPFSNSTNNGLLFINTTIASIAAKEEGVSLEKREAEA

SEQ ID NO: 22 - protein, 516 aa, Artificial Sequence; identical to SEQ ID NO: 2
  Col45opt hydroxyproline
  MOD_RES (5)..(5): 4Hyp
  MOD_RES (14)..(14): 4Hyp
  MOD_RES (26)..(26): 4Hyp
  MOD_RES (38)..(38): 4Hyp
  MOD_RES (41)..(41): 4Hyp
  MOD_RES (47)..(47): 4Hyp
  MOD_RES (53)..(53): 4Hyp
  MOD_RES (62)..(62): 4Hyp
  MOD_RES (80)..(80): 4Hyp
  MOD_RES (95)..(95): 4Hyp
  MOD_RES (101)..(101): 4Hyp
  MOD_RES (122)..(122): 4Hyp
  MOD_RES (128)..(128): 4Hyp
  MOD_RES (131)..(131): 4Hyp
  MOD_RES (140)..(140): 4Hyp
  MOD_RES (146)..(146): 4Hyp
  MOD_RES (164)..(164): 4Hyp
  MOD_RES (173)..(173): 4Hyp
  MOD_RES (182)..(182): 4Hyp
  MOD_RES (194)..(194): 4Hyp
  MOD_RES (200)..(200): 4Hyp
  MOD_RES (209)..(209): 4Hyp
  MOD_RES (218)..(218): 4Hyp
  MOD_RES (221)..(221): 4Hyp
  MOD_RES (242)..(242): 4Hyp
  MOD_RES (251)..(251): 4Hyp
  MOD_RES (260)..(260): 4Hyp
  MOD_RES (269)..(269): 4Hyp
  MOD_RES (287)..(287): 4Hyp
  MOD_RES (296)..(296): 4Hyp
  MOD_RES (299)..(299): 4Hyp
  MOD_RES (305)..(305): 4Hyp
  MOD_RES (320)..(320): 4Hyp
  MOD_RES (326)..(326): 4Hyp
  MOD_RES (332)..(332): 4Hyp
  MOD_RES (341)..(341): 4Hyp
  MOD_RES (347)..(347): 4Hyp
  MOD_RES (368)..(368): 4Hyp
  MOD_RES (371)..(371): 4Hyp
  MOD_RES (374)..(374): 4Hyp
  MOD_RES (443)..(443): 4Hyp
  MOD_RES (446)..(446): 4Hyp
  MOD_RES (449)..(449): 4Hyp
  MOD_RES (467)..(467): 4Hyp
  MOD_RES (482)..(482): 4Hyp
  MOD_RES (488)..(488): 4Hyp
  MOD_RES (503)..(503): 4Hyp
  MOD_RES (506)..(506): 4Hyp
  MOD_RES (509)..(509): 4Hyp
  MOD_RES (512)..(512): 4Hyp
  MOD_RES (515)..(515): 4Hyp

SEQ ID NO: 23 - DNA, 729 bp, Artificial Sequence
  Native P4H, L593
atgaaaactgtgactatcattacaataattgttgtaattattgttgttattttgattataatggtattgtcaaaatcttgtgtgtcccattttagaaatgtcggtagtttgaattcacgggatgtgaatttaaaagatgatttttcgtacgccaatattgatgatccttataataaaccatttgttttgaataatttgattaatccgaccaaatgtcaagaaattatgcaatttgccaatggaaaactttttgattcacaagttttaagtggtactgataaaaatattcgcaatagtcaacaaatgtggatatctaaaaataatcctatggtcaaacctatttttgaaaatatatgtagacaatttaatgttccatttgataatgctgaagatttgcaagttgttcgttatttacctaatcaatattataatgaacaccatgattcatgctgtgatagtagtaaacaatgtagtgaatttattgaaagaggtggtcaaagaattctaaccgtactaatttatctcaataatgaattttctgatggtcatacttatttccctaatttgaatcaaaaattcaaaccaaaaacaggagatgcactagtattttaccctttagctaataatagtaataaatgtcatccatattctttacatgctggaatgcctgttactagtggagaaaaatggattgccaatttatggtttagagaacgaaaattttcctaa

SEQ ID NO: 24 - protein, 242 aa, Artificial Sequence
  Native P4H, L593
MKTVTIITIIVVIIVVILIIMVLSKSCVSHFRNVGSLNSRDVNLKDDFSYANIDDPYNKPFVLNNLINPTKCQEIMQFANGKLFDSQVLSGTDKNIRNSQQMWISKNNPMVKPIFENICRQFNVPFDNAEDLQVVRYLPNQYYNEHHDSCCDSSKQCSEFIERGGQRILTVLIYLNNEFSDGHTYFPNLNQKFKPKTGDALVFYPLANNSNKCHPYSLHAGMPVTSGEKWIANLWFRERKFS

SEQ ID NO: 25 - DNA, 765 bp, Artificial Sequence
  P4H in pAOX_Mimi-int 3.0
atgaggcaggtttggttctcttggattgtgggattgttcctatgttttttcaacgtgtcttctgctcatcatcaccaccatcacatggttctgtccaaatcctgtgtttcacacttccgaaatgtaggttctctaaacagtagagatgttaatcttaaagacgatttcagctatgccaatattgatgatccttacaataagccatttgtgcttaataacctgattaaccctactaagtgtcaagaaatcatgcaatttgcaaatggcaagttgtttgattcacaggttttgtctgggactgacaagaacattagaaactcgcaacaaatgtggattagcaagaacaatcctatggtaaagccaatctttgagaatatttgcagacagttcaatgttccctttgacaatgctgaagatttgcaagtcgttcgttatcttccaaaccagtactataacgaacaccatgactcgtgttgtgactcttcaaaacaatgcagtgagttcattgagagaggtggtcaaaggattttgacagtcttgatctacctaaacaatgagttcagtgatggacacacttactttccgaacttaaaccagaaattcaagcccaaaactggagatgcattagtcttttatccattggccaataactctaacaaatgccatccatactccttacatgctggtatgcctgtaacatctggagaaaagtggattgctaatttgtggtttagagaacgtaaattctcccatgatgaattgtaa

SEQ ID NO: 26 - protein, 254 aa, Artificial Sequence
  P4H in pAOX_Mimi-int 3.0 1-22 Ost1, 23-28 His-Tag, 29-250 P4H, 251-254 retention signal
MRQVWFSWIVGLFLCFFNVSSAHHHHHHMVLSKSCVSHFRNVGSLNSRDVNLKDDFSYANIDDPYNKPFVLNNLINPTKCQEIMQFANGKLFDSQVLSGTDKNIRNSQQMWISKNNPMVKPIFENICRQFNVPFDNAEDLQVVRYLPNQYYNEHHDSCCDSSKQCSEFIERGGQRILTVLIYLNNEFSDGHTYFPNLNQKFKPKTGDALVFYPLANNSNKCHPYSLHAGMPVTSGEKWIANLWFRERKFSHDEL